European Patent Specification EP 3 353 316 B1, published January 10, 2024. Title: Methods of Prediction of Wound Healing. Applicant: Bayliff, Simon Brosnan, Patrick. The sequence listing filed with the application follows.

SEQUENCE LISTING (1 sequence)

SEQ ID NO: 1 - protein, 4 aa, Artificial
  Synthetic sequence
  MOD_RES (1)..(1): N-methylsuccinylalanine
  MOD_RES (4)..(4): Valine chloromethyl ketone
XAPX